European Patent Application EP 4 494 645 A1, published January 22, 2025. Title: A novel use of genetically modified oncolytic measles virus. Applicant: The University of Tokyo. Application JP. The sequence listing filed with the application follows.

SEQUENCE LISTING (12 sequences)

SEQ ID NO: 1 - DNA, 15894 bp, Measles virus
  source 1..15894: mol_type = genomic DNA
  CDS 108..1685
  CDS 1807..3330
  CDS 3438..4445
  CDS 5458..7110
  CDS 7271..9124
  CDS 9234..15785
accaaacaaagttgggtaaggatagatcaatcaatgatcatattctagtacacttaggattcaagatcctattatcagggacaagagcaggattagggatatccgagatggccacacttttgaggagcttagcattgttcaaaagaaacaaggacaaaccacccattacatcaggatccggtggagccatcagaggaatcaaacacattattatagtaccaattcctggagattcctcaattaccactcgatccaggctactggaccggttggtcaggttaattggaaacccggatgtgagcgggcccaaactaacaggggcactcataggtatattatccttatttgtggagtctccaggtcaattgattcagaggatcaccgatgaccctgacgttagcatcaggctgttagaggttgttcagagtgaccagtcacaatctggccttaccttcgcatcaagaggtaccaacatggaggatgaggcggaccaatacttttcacatgatgatccaagcaatagtgatcaatccaggtccggatggttcgagaacaaggaaatctcagatattgaagtgcaagaccctgagggattcaacatgattctgggtaccattctagcccagatctgggtcttgctcgcaaaggcggttacggccccagacacggcagctgattcggagctaagaaggtggataaagtacacccaacaaagaagggtagttggtgaatttagattggagagaaaatggttggatgtggtgaggaacaggattgccgaggacctctctttacgccgattcatggtggctctaatcctggatatcaagaggacacccgggaacaaacctaggattgctgaaatgatatgtgacattgatacatatatcgtagaggcaggattagccagttttatcctgactattaagtttgggatagaaactatgtatcctgctcttggactgcatgaatttgctggtgagttatccacacttgagtccttgatgaatctttaccagcaaatgggagaaactgcaccctacatggtaatcctagagaactcaattcagaacaagttcagtgcaggatcataccctctgctctggagctatgccatgggagtaggagtggaacttgaaaactccatgggaggtttgaactttggtcgatcttactttgatccagcatattttagattagggcaagagatggtgaggaggtcagctggaaaggtcagttccacattggcatccgaactcggtatcactgccgaggatgcaaggcttgtttcagagattgcaatgcatactactgaggacaggatcagtagagcggtcggacccagacaagcccaagtgtcatttctacacggtgatcaaagtgagaatgagctaccaggattggggggcaaggaagataggagggtcaaacagggtcggggagaagccagggagaactacagagaaaccgggtccagcagagcaagtgatgcgagagctgcccatcctccaaccagcatgcccctagacattgacactgcatcggagtcaggccaagatccgcaggacagtcaaaggtcagctgacgccctgctcaggctgcaagccatggcaggaatcttggaagaacaaggctcagacacggacacccctagggtatacaatgacagagatcttctagactaggtgcgagaggccgaggaccagaacaacatccacctaccctccatcattgttataaaaaacttaggaaccaggtccacacagccgccagccaaccaaccatccactcccacgactggagccaatggcagaagagcaggcacgccatgtcaaaaacggactggaatgcatccgggctctcaaggccgagcccatcggctcactggccgtcgaggaagccatggcagcatggtcagaaatatcagacaacccaggacaggaccgagccacctgcaaggaagaggaggcaggcagttcgggtctcagcaaaccatgcctctcagcaattggatcaactgaaggcggtgcacctcgcatccgcggtcagggatctggagaaagcgatgacgacgctgaaactttgggaatcccctcaagaaatctccaggcatcaagcactgggttacagtgttatcatgtttatgatcacagcggtgaagcggttaagggaatccaagatgctgactctatcatggttcaatcaggccttgatggtgatagcaccctctcaggaggagacgatgaatctgaaaacagcgatgtggatcttggcgaacctgataccgagggatatgctatcactgaccggggatctgctcccatctctatggggttcagggcttctgatgttgaaactgcagaaggaggggagatccacgagctcctgaaactccaatccagaggcaacaactttccgaagcttgggaaaactctcaatgttcctccgcccccgaaccccagtagggccagcacttccgagacacccattaaaaaggggacagacgcgagattggcctcatttggaacggagatcgcgtctttattgacaggtggtgcaacccaatgtgctcgaaagtcaccctcggaaccatcagggccaggtgcacctgcggggaatgtccccgagtgtgtgagcaatgccgcactgatacaggagtggacacccgaatctggtaccacaatctccccgagatcccagaataatgaagaagggggagactattatgatgatgagctgttctccgatgtccaagacatcaaaacagccttggccaaaatacacgaggataatcagaagataatctccaagctagaatcattgctgttattgaagggagaagttgagtcaatcaagaagcagatcaacaggcaaaatatcagcatatccaccctggaaggacacctctcaagcatcatgattgccattcctggacttgggaaggatcccaacgaccccaccgcagatgtcgaactcaatcccgacctgaaacccatcataggcagagattcaggccgagcactggccgaagttctcaagaagcccgttgccagccgacaactccagggaatgactaatggacggaccagttccagaggacagctgctgaaggaatttcaactaaagccgatcgggaaaaaggtgagctcagccgtcgggtttgttcctgacaccggccctgcatcacgcagtgtaatccgctccattataaaatccagccggctagaggaggatcggaagcgttacctgatgactctccttgatgatatcaaaggagccaacgatcttgccaagttccaccagatgctgatgaagataataatgaagtagctacagctcaacttacctgccaaccccatgccagtcgacctaattagtacaacctaaatccattataaaaaacttaggagcaaagtgattgcctcctaagttccacaatgacagagatctacgatttcgacaagtcggcatgggacatcaaagggtcgatcgctccgatacaacctaccacctacagtgatggcaggctggtgccccaggtcagagtcatagatcctggtctaggtgataggaaggatgaatgctttatgtacatgtttctgctgggggttgttgaggacagcgatcccctagggcctccaatcgggcgagcattcgggtccctgcccttaggtgttggtagacccacagcaaaacccgaggaactcctcaaagaggccactgagcttgacatagttgttagacgtacagcagggctcaatgaaaaactggtgttctacaacaacaccccactaaccctcctcacaccttggagaaaggtcctaacaacagggagtgtcttcaatgcaaaccaagtgtgcaatgcggttaatctaataccgctggacaccccgcagaggttccgtgttgtttatatgagcatcacccgtctttcggataacgggtattacaccgttcccagaagaatgctggaattcagatcggtcaatgcagtggccttcaacctgctagtgacccttaggattgacaaggcaattggccctgggaagatcatcgacaatgcagagcaacttcctgaggcaacatttatggtccacatcgggaacttcaggagaaagaagagtgaagtctactctgccgattattgcaaaatgaaaatcgaaaagatgggcctggtttttgcacttggtgggatagggggcaccagtcttcacattagaagcacaggcaaaatgagcaagactctccatgcacaactcgggttcaagaagaccttatgttacccactgatggatatcaatgaagaccttaatcggttactctggaggagcagatgcaagatagtaagaatccaggcagttttgcagccatcagttcctcaagaattccgcatttacgacgacgtgatcataaatgatgaccaaggactattcaaagttctgtagaccgcagtgcccagcaatacccgaaaacgacccccctcataatgacagccagaaggcccggacaaaaaagccccctccagaagactccacggaccaagcgagaggccagccagcagccgacagcaagtgtggacaccaggcggcccaagcacagaacagccccgacacaaggccaccaccagccatcccaatctgcgtcctcctcgtgggacccccgaggaccaatcctgaaggtcgctccgaacacagaccaccaaccgcatccccacagctcccgggaaaggaacccccagcaattggaaggcccctccccccctcccccaacgcaagaaccccacaaccgaaccgcacaagcgaccgaggtgacccaaccgcaggcatccgactccttagacagatcctctccccccggcatactaaacaaaacttagggccaaggaacacacacacccgacagaacccagaccccggcccgcggcaccgcgcccccaccccccgaaaaccagagggagcccccaaccaaacccgccggcccccccggtgcccacaggtaggcacaccgacccccgaccagacccagcacccagccaccgacaatccaagacggggggccccccccaaaaaaaggcccccaggggccgacagccagcatcgcgaggaagcacacccaccccacacacgaccacggcaaccgaaccagagtccagaccaccctgggccaccagctcccagactcggccatcaccccgcaaaaaggaaaggccacaacccgcgcaccccagccccgatccggcgggcagccactcaacccgaaccagcacccaagagcgatccttgggggacccccaaaccgcaaaagacatcagtatcccacagcctctccaagtcccccggtctcctcctcttctcgaagggaccaaaagatcaatccaccacatccgacgacactcaatttcccacccccaaaggagacaccgggaatcccagaatcaagactcatccagtgtccatcatgggtctcaaggtgaacgtctctgccatattcatggcagtactgttaactctccaaacacccaccggtcaaatccattggggcaatctctctaagataggggtggtagggataggaagtgcaagctacaaagttatgactcgttccagccatcaatcattggtcataaaattaatgcccaatataactctcctcaataactgcacgagggtagagatcgcagaatacaggagactactgagaacagttttggaaccaattagagatgcacttaatgcaatgacccagaatataagaccggttcagagtgtagcttcaagtaggagacacaagagatttgcgggagtagtcctggcaggtgcggccctaggcgttgccacagctgctcagataacagccggcattgcacttcatcagtccatgctgaactctcaagccatcgacaatctgagagcgagcctggaaactactaatcaggcaattgaggcaatcagacaagcagggcaggagatgatattggctgctcagggtgtccaagactacatcaataatgagctgataccgtctatgaaccaactatcttgtgatttaatcggccagaagctagggctcaaattgctcagatactatacagaaatcctgtcattatttggccccagcttacgggaccccatatctgcggagatatccatccaggcttcgagctatgcgcttggaggagatatcaataaggtgttagaaaagctcggatacagtggaggtgatttactgggcatcttagagagcaggggaataaaggcccggataactcacgtcgacacagagtcctacttcattgtactcagtatagcctatccgacgctgtccgagattaagggggtgattgtccaccggctagagggggtctcgtacaatataggctctcaagagtggtataccactgtgcccaagtatgttgcaacccaagggtaccttatctcgaattttgatgagtcatcgtgtactttcatgccagaggggactgtgtgcagccaaaatgccttgtacccgatgagtcctctgctccaagaatgcctccgggggtccaccaagtcctgtgctcgtacactcgtatccgggtcttttgggaaccggttcattttatcacaagggaacctaatagccaattgtgcatcaatcctctgcaagtgttacacaacaggaacgatcattaatcaagaccctgacaagatcctaacatacattgctgccgatcactgcccggtggtcgaggtgaacggcgtgaccatccaagtcgggagcaggaggtatccggacgcggtgtacctgcacagaattgacctcggtcctcccatatcattggagaggttggacgtagggacaaatctggggaatgcaattgctaagttggaggatgccaaggaattgttggagtcatcggaccagatattgaggagtatgaaaggtttatcgagcactagcatagtttacatcctgattgcagtgtgtcttggagggttgatagggatccccgctttaatatgttgctgcagggggcgctgtaacaaaaagggagaacaagttggtatgtcaagaccaggcctaaagcctgatcttacggggacatcaaaatcctatgtaaggtcgctctgatcctctacaactcttgaaacacagatttcccacaagtctcctcttcgtcatcaagcaaccaccgcatccagcatcaagcccacttgaaattgtctccggcttccctctggccgaacgatatcggtagttaattaaaacttagggtgcaagatcatccacaatgtcaccacaacgagaccgaataaatgccttctacaaagacaacccacatcctaagggaagtaggatagttattaacagagaacatcttatgattgatagaccttatgttttgctggctgttctattcgtcatgtttctgagcttgatcgggttgctagccatcgcaggcattagactccatcgtgcagccatctacaccgcagagatccataagagcctcagcaccaatctagatgtaactaactcaatcgagcatcaggtcaaggacgtgctgacaccactcttcaagatcattggtgatgaagtgggcctgaggacacctcagagattcactgacctagtgaaattcatctctgacaaaattaaattccttaatccggatagggagtacgacttcagagatctcacttggtgtatcaacccgccagagagaatcaaattggattatgatcaatactgtgcagatgtggctgctgaagaactcatgaatgcattggtgaactcaactctactggaggccagggcaaccaatcagttcctagctgtctcaaagggaaactgctcagggcccactacaatcagaggtcaattctcaaacatgtcgctgtccctgttggacttgtatttaagtcgaggttacaatgtatcgtctatagtcactatgacatcccagggaatgtacgggggaacttacctagtggaaaagcctaatctgagcagtaaagggtcagagttgtcacaactgagcatgcaccgagtgtttgaagtaggggttatcagaaatccgggtttgggggctccggtgttccatatgacaaactattttgagcaaccagtcagtaatgatttcagcaactgcatggtggctttgggggagcttaaattcgcagccctctgtcacagggaagattctatcacaattccctatcaggggtcagggaaaggtgtcagcttccagctcgtcaagctaggtgtctggaaatccccaactgacatgcgatcctgggtccccctatcaacggatgatccagtgatagataggctttacctctcatctcacagaggtgttatcgctgacaatcaagcaaaatgggctgtcccgacaacacggacagatgacaagttgcgaatggagacatgcttccagcaggcgtgtaagggtaaaaaccaagcactctgcgagaatcccgagtgggcaccattgaaggataacaggattccttcatacggggtcttgtctgttaatctgagtctgacagctgagcttaaaatcaaaattgcttcaggattcgggccattgatcacacacggttcagggatggacctatacaaaaccaaccacaacaatgtgtattggctgactatcccgccaatgaagaacttagccttaggtgtaatcaacacattggagtggataccgagattcaaggttagtcccaacctcttcactgttccaatcaaggaagcaggcgaggactgccatgccccaacatacctacctgcggaggtggatggtgatgtcaaactcagttccaatctggtaattctacctggtcaggatctccaatatgttttggcaacctacgatacttccgcagttgaacatgctgtggtttattatgtttacagcccaagccgctcattttcttacttttatccttttaggttgcctataaagggggtcccaatcgaattacaagtggaatgcttcacatgggacaaaaaactctggtgccgtcacttctgtgtgcttgcggactcagaatctggtggacatatcactcactctgggatggtgggcatgggagtcagctgcacagtcactcgggaagatggaaccaatcgcagatagggctgccagtgaaccgatcacatgatgtcacccagacatcaggcatacccactagtgtgaaatagacatcagaattaagaaaaacgtagggtccaagtggtttcccgttatggactcgctatctgtcaaccagatcttataccctgaagttcacctagatagcccgatagttaccaataagatagtagctatcctggagtatgctcgagtccctcacgcttacagcctggaggaccctacactgtgtcagaacatcaagcaccgcctaaaaaacggattctccaaccaaatgattataaacaatgtggaagttgggaatgtcatcaagtccaagcttaggagttatccggcccactctcatattccatatccaaattgtaatcaggatttatttaacatagaagacaaagagtcaacaaggaagatccgtgagctcctaaaaaagggaaattcgctgtactccaaagtcagtgataaggttttccaatgcctgagggacactaactcacggcttggcctaggctccgaattgagggaggacatcaaggagaaaattattaacttgggagtttacatgcacagctcccaatggtttgagccctttctgttttggtttacagtcaagactgagatgaggtcagtgattaaatcacaaacccatacttgccataggaggagacacacacctgtattcttcactggtagttcagttgagctgttaatctctcgtgaccttgttgctataatcagtaaggagtctcaacatgtatattacctgacgtttgaactggttttgatgtattgtgatgtcatagaggggaggttaatgacagagaccgctatgaccattgatgctaggtatgcagaacttctaggaagagtcagatacatgtggaaactgatagatggtttcttccctgcactcgggaatccaacttatcaaattgtagccatgctggagccactttcacttgcttacctgcaactgagggatataacagtagaactcagaggtgctttccttaaccactgctttactgaaatacatgatgttcttgaccaaaacgggttttctgatgaaggtacttatcatgagttaattgaagccctagattacattttcataactgatgacatacatctgacaggggagattttctcatttttcagaagtttcggccaccccagacttgaagcagtaacggctgctgaaaatgtcaggaaatacatgaatcagcctaaagtcattgtgtatgagactctgatgaaaggtcatgccatattttgtggaatcataatcaacggctatcgtgacaggcacggaggcagttggccacccctgaccctccccctgcatgctgcagacacaatccggaatgctcaagcttcaggtgaagggttaacacatgagcagtgcgttgataactggaaatcatttgctggagtgagatttggctgttttatgcctcttagcctggacagtgatctgacaatgtacctaaaggacaaggcacttgctgctctccaaagggaatgggattcagtttacccgaaagagttcctgcgttacgatcctcccaagggaaccgggtcacggaggcttgtagatgttttccttaatgattcgagctttgacccatatgatatgataatgtatgtcgtaagtggagcctacctccatgaccctgagttcaacctgtcttacagcctgaaagaaaaggagatcaaggaaacaggtagacttttcgctaaaatgacttacaaaatgagggcatgccaagtgatcgctgaaaatctaatctcaaacgggattggcaagtattttaaggacaatgggatggccaaggatgagcacgatttgactaaggcactccacactctggctgtctcaggagtccccaaagatctcaaagaaagtcacaggggggggccagtcttaaaaacctactcccgaagcccagtccacacaagtaccaggaacgttaaagcaaaaaaagggtttgtaggattccctcatgtaattcggcagaatcaagacactgatcatccggagaatatagaaacctacgagacagtcagcgcatttatcacgactgatctcaagaagtactgccttaattggagatatgagaccatcagcttatttgcacagaggctaaatgagatttacggattaccctcattttttcagtggctgcataagaggcttgaaacctctgtcctctatgtaagtgaccctcattgcccccccgaccttgacgcccatgtcccgttatgcaaagtccccaatgaccaaatcttcatcaagtaccctatgggaggtatagaagggtattgtcagaagctgtggaccatcagcaccattccctacttatacctggctgcttatgagagcggggtaaggattgcttcgttagtgcaaggggacaatcagaccatagccgtaacaaaaagggtacccagcacatggccttacaaccttaagaaacgggaagctgctagagtaactagagattactttgtaattcttaggcaaaggctacatgacattggccatcacctcaaggcaaatgagacaattgtttcatcacatttttttgtctattcaaaaggaatatattatgatgggctacttgtgtcccaatcactcaagagcatcgcaagatgtgtattctggtcagagactatagttgatgaaacaagggcagcatgcagtaatattgctacaacaatggctaaaagcatcgagagaggttatgaccgttatcttgcatattccctgaacgtcctaaaagtgatacagcaaattttgatctctcttggcttcacaatcaattcaaccatgacccgagatgtagtcatacccctcctcacaaacaacgatctcttaataaggatggcactgttgcccgctcctattggggggatgaattatctgaatatgagcaggctgtttgtcagaaacatcggtgatccagtaacatcatcaattgctgatctcaagagaatgattctcgcatcactaatgcctgaagagaccctccatcaagtaatgacacaacaaccgggggactcttcattcctagactgggctagcgacccttactcagcaaatcttgtatgcgtccagagcatcactagactcctcaagaacataactgcaaggtttgtcctaatccatagtccaaacccaatgttaaaagggttattccatgatgacagtaaagaagaggacgagagactggcggcattcctcatggacaggcatattatagtacctagggcagctcatgaaatcctggatcatagtgtcacaggggcaagagagtctattgcaggcatgctagataccacaaaaggcctgattcgagccagcatgaggaagggggggttaacctctcgagtgataaccagattgtccaattatgactatgaacaatttagagcagggatggtgctattgacaggaagaaagagaaatgtcctcattgacaaagagtcatgttcagtgcagctggctagagccctaagaagccatatgtgggcaagactagctcgaggacggcctatttacggccttgaggtccctgatgtactagaatctatgcgaggccaccttattcggcgtcatgagacatgtgtcatctgcgagtgtggatcagtcaactacggatggttttttgtcccctcgggttgccaactggatgatattgacaaggaaacatcatccttgagagtcccatatattggttctaccactgatgagagaacagacatgaagctcgcattcgtaagagccccaagtagatccttgcgatctgccgttagaatagcaacagtgtactcatgggcttacggtgatgatgatagctcttggaacgaagcctggttgttggcaaggcaaagggccaatgtgagcctggaggagctaagggtgatcactcccatctcgacttcgactaatttagcgcataggttgagggatcgtagcactcaagtgaaatactcaggtacatcccttgtccgagtggcaaggtataccacaatctccaacgacaatctctcatttgtcatatcagataagaaggttgatactaactttatataccaacaaggaatgcttctagggttgggtgttttagaaacattgtttcgactcgagaaagatactggatcatctaacacggtattacatcttcacgtcgaaacagattgttgcgtgatcccgatgatagatcatcccaggatacccagctcccgcaagctagagctgagggcagagctatgtaccaacccattgatatatgataatgcacctttaattgacagagatgcaacaaggctatacacccagagccataggaggcaccttgtggaatttgttacatggtccacaccccaactatatcacattctagctaagtccacagcactatctatgattgacctggtaacaaaatttgagaaggaccatatgaatgaaatttcagctctcataggggatgacgatatcaatagtttcataactgagtttctgcttatagagccaagattattcaccatctacttgggccagtgtgcagccatcaattgggcatttgatgtacattatcatagaccatcagggaaatatcagatgggtgagctgttgtcttcgttcctttctagaatgagcaaaggagtgtttaaggtgcttgtcaatgctctaagccacccaaagatctacaagaaattctggcattgtggtattatagagcctatccatggtccttcacttgatgctcaaaacttgcacacaactgtgtgcaacatggtttacacatgctatatgacctacctcgacctgttgttgaatgaagagttagaagagttcacatttcttttgtgtgaaagcgatgaggatgtagtaccggacagattcgacaacatccaggcaaaacacttgtgtgttctggcagatttgtactgtcaaccggggacctgcccaccgattcgaggtctaaggccggtagagaaatgtgcagttctaaccgatcatatcaagacagaggctaggttatctccagcaggatcttcgtggaacataaatccaattattgtagaccattactcatgctctctgacttatctccgtcgaggatctatcaaacagataagattgagagttgatccaggattcatttttgacgccctcgctgaggtaaatgtcagtcagccaaaggtcggcagcaacaacatctcaaatatgagcatcaaggatttcagacctccacacgatgatgttgcaaaattgctcaaagatatcaacacaagcaagcacaatcttcccatttcagggggtagtctcgccaattatgaaatccatgctttccgcagaatcgggttaaactcatctgcttgctacaaagctgttgagatatcaacattaattaggagatgccttgagccaggggaagacggcttgttcttgggtgaggggtcgggttctatgttgatcacttataaggagatactaaaactaaacaagtgcttctataatagtggggtttccgccaattctagatctggtcaaagggaattagcaccctatccctccgaagttggccttgtcgaacacagaatgggagtaggtaatattgtcaaggtgctctttaacgggaggcccgaagtcacgtgggtaggcagtatagattgcttcaatttcatagtcagtaatatccctacctctagtgtggggtttatccattcagatatagagaccttacctaacaaagatactatagagaagctagaggaattggcagccatcttatcgatggctctactccttggcaaaataggatcaatactggtgattaagcttatgcctttcagcggggattttgttcagggatttataagctatgtagggtctcattatagagaagtgaaccttgtctaccctaggtacagcaacttcatatctactgaatcttatttagttttgacagatctcaaagctaaccggctaatgaatcctgaaaagatcaagcagcagataattgaatcatctgtgcggacttcacctggacttataggtcacatcctatccattaagcaactaagctgcatacaagcaattgtgggaggcgcagttagtagaggtgatatcaaccctattctgaaaaaacttacacctatagagcaggtgctgatcagttgcgggttggcaattaacggacctaaactgtgcaaagaattaatccaccatgatgttgcctcagggcaagatggattgcttaactctatactcatcctctacagggagttggcaagattcaaagacaaccaaagaagtcaacaagggatgttccacgcttaccccgtattggtaagtagtaggcaacgagaacttgtatctaggatcactcgcaaattttgggggcatattcttctttactccgggaacagaaagttgataaatcggtttatccagaatctcaagtccggttatctagtactagacttacaccagaatatcttcgttaagaatctatccaagtcagagaaacagattattatgacggggggtttaaaacgtgagtgggtttttaaggtaacagtcaaggagaccaaagaatggtacaagttagtcggatacagcgctctgattaaggattaattggttgaactccggaaccctaatcctgccctaggtagttaggcattatttgcaatatattaaagaaaactttgaaaatacgaagtttctattcccagctttgtctggt

SEQ ID NO: 2 - protein, 525 aa, Measles virus
MATLLRSLALFKRNKDKPPITSGSGGAIRGIKHIIIVPIPGDSSITTRSRLLDRLVRLIGNPDVSGPKLTGALIGILSLFVESPGQLIQRITDDPDVSIRLLEVVQSDQSQSGLTFASRGTNMEDEADQYFSHDDPSNSDQSRSGWFENKEISDIEVQDPEGFNMILGTILAQIWVLLAKAVTAPDTAADSELRRWIKYTQQRRVVGEFRLERKWLDVVRNRIAEDLSLRRFMVALILDIKRTPGNKPRIAEMICDIDTYIVEAGLASFILTIKFGIETMYPALGLHEFAGELSTLESLMNLYQQMGETAPYMVILENSIQNKFSAGSYPLLWSYAMGVGVELENSMGGLNFGRSYFDPAYFRLGQEMVRRSAGKVSSTLASELGITAEDARLVSEIAMHTTEDRISRAVGPRQAQVSFLHGDQSENELPGLGGKEDRRVKQGRGEARENYRETGSSRASDARAAHPPTSMPLDIDTASESGQDPQDSQRSADALLRLQAMAGILEEQGSDTDTPRVYNDRDLLD

SEQ ID NO: 3 - protein, 507 aa, Measles virus
MAEEQARHVKNGLECIRALKAEPIGSLAVEEAMAAWSEISDNPGQDRATCKEEEAGSSGLSKPCLSAIGSTEGGAPRIRGQGSGESDDDAETLGIPSRNLQASSTGLQCYHVYDHSGEAVKGIQDADSIMVQSGLDGDSTLSGGDDESENSDVDLGEPDTEGYAITDRGSAPISMGFRASDVETAEGGEIHELLKLQSRGNNFPKLGKTLNVPPPPNPSRASTSETPIKKGTDARLASFGTEIASLLTGGATQCARKSPSEPSGPGAPAGNVPECVSNAALIQEWTPESGTTISPRSQNNEEGGDYYDDELFSDVQDIKTALAKIHEDNQKIISKLESLLLLKGEVESIKKQINRQNISISTLEGHLSSIMIAIPGLGKDPNDPTADVELNPDLKPIIGRDSGRALAEVLKKPVASRQLQGMTNGRTSSRGQLLKEFQLKPIGKKVSSAVGFVPDTGPASRSVIRSIIKSSRLEEDRKRYLMTLLDDIKGANDLAKFHQMLMKIIMK

SEQ ID NO: 4 - protein, 335 aa, Measles virus
MTEIYDFDKSAWDIKGSIAPIQPTTYSDGRLVPQVRVIDPGLGDRKDECFMYMFLLGVVEDSDPLGPPIGRAFGSLPLGVGRPTAKPEELLKEATELDIVVRRTAGLNEKLVFYNNTPLTLLTPWRKVLTTGSVFNANQVCNAVNLIPLDTPQRFRVVYMSITRLSDNGYYTVPRRMLEFRSVNAVAFNLLVTLRIDKAIGPGKIIDNAEQLPEATFMVHIGNFRRKKSEVYSADYCKMKIEKMGLVFALGGIGGTSLHIRSTGKMSKTLHAQLGFKKTLCYPLMDINEDLNRLLWRSRCKIVRIQAVLQPSVPQEFRIYDDVIINDDQGLFKVL

SEQ ID NO: 5 - protein, 550 aa, Measles virus
MGLKVNVSAIFMAVLLTLQTPTGQIHWGNLSKIGVVGIGSASYKVMTRSSHQSLVIKLMPNITLLNNCTRVEIAEYRRLLRTVLEPIRDALNAMTQNIRPVQSVASSRRHKRFAGVVLAGAALGVATAAQITAGIALHQSMLNSQAIDNLRASLETTNQAIEAIRQAGQEMILAAQGVQDYINNELIPSMNQLSCDLIGQKLGLKLLRYYTEILSLFGPSLRDPISAEISIQASSYALGGDINKVLEKLGYSGGDLLGILESRGIKARITHVDTESYFIVLSIAYPTLSEIKGVIVHRLEGVSYNIGSQEWYTTVPKYVATQGYLISNFDESSCTFMPEGTVCSQNALYPMSPLLQECLRGSTKSCARTLVSGSFGNRFILSQGNLIANCASILCKCYTTGTIINQDPDKILTYIAADHCPVVEVNGVTIQVGSRRYPDAVYLHRIDLGPPISLERLDVGTNLGNAIAKLEDAKELLESSDQILRSMKGLSSTSIVYILIAVCLGGLIGIPALICCCRGRCNKKGEQVGMSRPGLKPDLTGTSKSYVRSL

SEQ ID NO: 6 - protein, 617 aa, Measles virus
MSPQRDRINAFYKDNPHPKGSRIVINREHLMIDRPYVLLAVLFVMFLSLIGLLAIAGIRLHRAAIYTAEIHKSLSTNLDVTNSIEHQVKDVLTPLFKIIGDEVGLRTPQRFTDLVKFISDKIKFLNPDREYDFRDLTWCINPPERIKLDYDQYCADVAAEELMNALVNSTLLEARATNQFLAVSKGNCSGPTTIRGQFSNMSLSLLDLYLSRGYNVSSIVTMTSQGMYGGTYLVEKPNLSSKGSELSQLSMHRVFEVGVIRNPGLGAPVFHMTNYFEQPVSNDFSNCMVALGELKFAALCHREDSITIPYQGSGKGVSFQLVKLGVWKSPTDMRSWVPLSTDDPVIDRLYLSSHRGVIADNQAKWAVPTTRTDDKLRMETCFQQACKGKNQALCENPEWAPLKDNRIPSYGVLSVNLSLTAELKIKIASGFGPLITHGSGMDLYKTNHNNVYWLTIPPMKNLALGVINTLEWIPRFKVSPNLFTVPIKEAGEDCHAPTYLPAEVDGDVKLSSNLVILPGQDLQYVLATYDTSAVEHAVVYYVYSPSRSFSYFYPFRLPIKGVPIELQVECFTWDKKLWCRHFCVLADSESGGHITHSGMVGMGVSCTVTREDGTNRR

SEQ ID NO: 7 - protein, 2183 aa, Measles virus
MDSLSVNQILYPEVHLDSPIVTNKIVAILEYARVPHAYSLEDPTLCQNIKHRLKNGFSNQMIINNVEVGNVIKSKLRSYPAHSHIPYPNCNQDLFNIEDKESTRKIRELLKKGNSLYSKVSDKVFQCLRDTNSRLGLGSELREDIKEKIINLGVYMHSSQWFEPFLFWFTVKTEMRSVIKSQTHTCHRRRHTPVFFTGSSVELLISRDLVAIISKESQHVYYLTFELVLMYCDVIEGRLMTETAMTIDARYAELLGRVRYMWKLIDGFFPALGNPTYQIVAMLEPLSLAYLQLRDITVELRGAFLNHCFTEIHDVLDQNGFSDEGTYHELIEALDYIFITDDIHLTGEIFSFFRSFGHPRLEAVTAAENVRKYMNQPKVIVYETLMKGHAIFCGIIINGYRDRHGGSWPPLTLPLHAADTIRNAQASGEGLTHEQCVDNWKSFAGVRFGCFMPLSLDSDLTMYLKDKALAALQREWDSVYPKEFLRYDPPKGTGSRRLVDVFLNDSSFDPYDMIMYVVSGAYLHDPEFNLSYSLKEKEIKETGRLFAKMTYKMRACQVIAENLISNGIGKYFKDNGMAKDEHDLTKALHTLAVSGVPKDLKESHRGGPVLKTYSRSPVHTSTRNVKAKKGFVGFPHVIRQNQDTDHPENIETYETVSAFITTDLKKYCLNWRYETISLFAQRLNEIYGLPSFFQWLHKRLETSVLYVSDPHCPPDLDAHVPLCKVPNDQIFIKYPMGGIEGYCQKLWTISTIPYLYLAAYESGVRIASLVQGDNQTIAVTKRVPSTWPYNLKKREAARVTRDYFVILRQRLHDIGHHLKANETIVSSHFFVYSKGIYYDGLLVSQSLKSIARCVFWSETIVDETRAACSNIATTMAKSIERGYDRYLAYSLNVLKVIQQILISLGFTINSTMTRDVVIPLLTNNDLLIRMALLPAPIGGMNYLNMSRLFVRNIGDPVTSSIADLKRMILASLMPEETLHQVMTQQPGDSSFLDWASDPYSANLVCVQSITRLLKNITARFVLIHSPNPMLKGLFHDDSKEEDERLAAFLMDRHIIVPRAAHEILDHSVTGARESIAGMLDTTKGLIRASMRKGGLTSRVITRLSNYDYEQFRAGMVLLTGRKRNVLIDKESCSVQLARALRSHMWARLARGRPIYGLEVPDVLESMRGHLIRRHETCVICECGSVNYGWFFVPSGCQLDDIDKETSSLRVPYIGSTTDERTDMKLAFVRAPSRSLRSAVRIATVYSWAYGDDDSSWNEAWLLARQRANVSLEELRVITPISTSTNLAHRLRDRSTQVKYSGTSLVRVARYTTISNDNLSFVISDKKVDTNFIYQQGMLLGLGVLETLFRLEKDTGSSNTVLHLHVETDCCVIPMIDHPRIPSSRKLELRAELCTNPLIYDNAPLIDRDATRLYTQSHRRHLVEFVTWSTPQLYHILAKSTALSMIDLVTKFEKDHMNEISALIGDDDINSFITEFLLIEPRLFTIYLGQCAAINWAFDVHYHRPSGKYQMGELLSSFLSRMSKGVFKVLVNALSHPKIYKKFWHCGIIEPIHGPSLDAQNLHTTVCNMVYTCYMTYLDLLLNEELEEFTFLLCESDEDVVPDRFDNIQAKHLCVLADLYCQPGTCPPIRGLRPVEKCAVLTDHIKTEARLSPAGSSWNINPIIVDHYSCSLTYLRRGSIKQIRLRVDPGFIFDALAEVNVSQPKVGSNNISNMSIKDFRPPHDDVAKLLKDINTSKHNLPISGGSLANYEIHAFRRIGLNSSACYKAVEISTLIRRCLEPGEDGLFLGEGSGSMLITYKEILKLNKCFYNSGVSANSRSGQRELAPYPSEVGLVEHRMGVGNIVKVLFNGRPEVTWVGSIDCFNFIVSNIPTSSVGFIHSDIETLPNKDTIEKLEELAAILSMALLLGKIGSILVIKLMPFSGDFVQGFISYVGSHYREVNLVYPRYSNFISTESYLVLTDLKANRLMNPEKIKQQIIESSVRTSPGLIGHILSIKQLSCIQAIVGGAVSRGDINPILKKLTPIEQVLISCGLAINGPKLCKELIHHDVASGQDGLLNSILILYRELARFKDNQRSQQGMFHAYPVLVSSRQRELVSRITRKFWGHILLYSGNRKLINRFIQNLKSGYLVLDLHQNIFVKNLSKSEKQIIMTGGLKREWVFKVTVKETKEWYKLVGYSALIKD

SEQ ID NO: 8 - DNA, 12 bp, synthetic construct
  source 1..12: mol_type = other DNA
accaaacaaagt

SEQ ID NO: 9 - DNA, 26 bp, synthetic construct
  source 1..26: mol_type = other DNA
caatcaatgatcatattctagtacac

SEQ ID NO: 10 - DNA, 25 bp, synthetic construct
  source 1..25: mol_type = other DNA
tataataatgtgtttgattcctctg

SEQ ID NO: 11 - DNA, 34 bp, synthetic construct
  source 1..34: mol_type = other DNA
aaaccggtgccaccatggaagacgccaaaaacat

SEQ ID NO: 12 - DNA, 28 bp, synthetic construct
  source 1..28: mol_type = other DNA
ttggatccttacacggcgatctttccgc